European Patent Application EP 4 585 682 A1, published July 16, 2025. Title: MUTATED V-TYPE CRISPR ENZYME AND USE THEREOF. Applicant: Beijing Synsortech Co., Ltd. Application CN. The sequence listing filed with the application follows.

SEQUENCE LISTING (21 sequences)

SEQ ID NO: 1 - protein, 1129 aa, synthetic construct
MAVKSMKVKLRLDNMPEIRAGLWKLHTEVNAGVRYYTEWLSLLRQENLYRRSPNGDGEQECYKTAEECKAELLERLRARQVENGHCGPAGSDDELLQLARQLYELLVPQAIGAKGDAQQIARKFLSPLADKDAVGGLGIAKAGNKPRWVRMREAGEPGWEEEKAKAEARKSTDRTADVLRALADFGLKPLMRVYTDSDMSSVQWKPLRKGQAVRTWDRDMFQQAIERMMSWESWNQRVGEAYAKLVEQKSRFEQKNFVGQEHLVQLVNQLQQDMKEASHGLESKEQTAHYLTGRALRGSDKVFEKWEKLDPDAPFDLYDTEIKNVQRRNTRRFGSHDLFAKLAEPKYQALWREDASFLTRYAVYNSIVRKLNHAKMFATFTLPDATAHPIWTRFDKLGGNLHQYTFLFNEFGEGRHAIRFQKLLTVEDGVAKEVDDVTVPISMSAQLDDLLPRDPHELVALYFQDYGAEQHLAGEFGGAKIQYRRDQLNHLHARRGARDVYLNLSVRVQSQSEARGERRPPYAAVFRLVGDNHRAFVHFDKLSDYLAEHPDDGKLGSEGLLSGLRVMSVDLGLRTSASISVFRVARKDELKPNSEGRVPFCFPIEGNENLVAVHERSQLLKLPGETESKDLRAIREERQRTLRQLRTQLAYLRLLVRCGSEDVGRRERSWAKLIEQPMDANQMTPDWREAFEDELQKLKSLYGICGDREWTEAVYESVRRVWRHMGKQVRDWRKDVRSGERPKIRGYQKDVVGGNSIEQIEYLERQYKFLKSWSFFGKVSGQVIRAEKGSRFAITLREHIDHAKEDRLKKLADRIIMEALGYVYALDDERGKGKWVAKYPPCQLILLEELSEYQFNNDRPPSENNQLMQWSHRGVFQELLNQAQVHDLLVGTMYAAFSSRFDARTGAPGIRCRRVPARCAREQNPEPFPWWLNKFVAEHKLDGCPLRADDLIPTGEGEFFVSPFSAEEGDFHQIHADLNAAQNLQRRLWSDFDISQIRLRCDWGEVDGEPVLIPRTTGKRTADSYGNKVFYTKTGVTYYERERGKKRRKVFAQEELSEEEAELLVEADEAREKSVVLMRDPSGIINRGDWTRQKEFWSMVNQRIEGYLVKQIRSRVRLQESACENTGDI

SEQ ID NO: 2 - protein, 767 aa, synthetic construct
MAQASSTPAVSPRPRPRYREERTLVRKLLPRPGQSKQEFRENVKKLRKAFLQFNADVSGVCQWAIQFRPRYGKPAEPTETFWKFFLEPETSLPPNDSRSPEFRRLQAFEAAAGINGAAALDDPAFTNELRDSILAVASRPKTKEAQRLFSRLKDYQPAHRMILAKVAAEWIESRYRRAHQNWERNYEEWKKEKQEWEQNHPELTPEIREAFNQIFQQLEVKEKRVRICPAARLLQNKDNCQYAGKNKHSVLCNQFNEFKKNHLQGKAIKFFYKDAEKYLRCGLQSLKPNVQGPFREDWNKYLRYMNLKEETLRGKNGGRLPHCKNLGQECEFNPHTALCKQYQQQLSSRPDLVQHDELYRKWRREYWREPRKPVFRYPSVKRHSIAKIFGENYFQADFKNSVVGLRLDSMPAGQYLEFAFAPWPRNYRPQPGETEISSVHLHFVGTRPRIGFRFRVPHKRSRFDCTQEELDELRSRTFPRKAQDQKFLEAARKRLLETFPGNAEQELRLLAVDLGTDSARAAFFIGKTFQQAFPLKIVKIEKLYEQWPNQKQAGDRRDASSKQPRPGLSRDHVGRHLQKMRAQASEIAQKRQELTGTPAPETTTDQAAKKATLQPFDLRGLTVHTARMIRDWARLNARQIIQLAEENQVDLIVLESLRGFRPPGYENLDQEKKRRVAFFAHGRIRRKVTEKAVERGMRVVTVPYLASSKVCAECRKKQKDNKQWEKNKKRGLFKCEGCGSQAQVDENAARVLGRVFWGEIELPTAIP

SEQ ID NO: 3 - protein, 26 aa, synthetic construct
CAREQNPEPFPWWLNKFVAEHKLDGC

SEQ ID NO: 4 - protein, 28 aa, synthetic construct
CARCRKKQKDNKQWEKNKKRGLFKCEGC

SEQ ID NO: 5 - protein, 1131 aa, synthetic construct
MAVKSMKVKLRLDNMPEIRAGLWKLHTEVNAGVRYYTEWLSLLRQENLYRRSPNGDGEQECYKTAEECKAELLERLRARQVENGHCGPAGSDDELLQLARQLYELLVPQAIGAKGDAQQIARKFLSPLADKDAVGGLGIAKAGNKPRWVRMREAGEPGWEEEKAKAEARKSTDRTADVLRALADFGLKPLMRVYTDSDMSSVQWKPLRKGQAVRTWDRDMFQQAIERMMSWESWNQRVGEAYAKLVEQKSRFEQKNFVGQEHLVQLVNQLQQDMKEASHGLESKEQTAHYLTGRALRGSDKVFEKWEKLDPDAPFDLYDTEIKNVQRRNTRRFGSHDLFAKLAEPKYQALWREDASFLTRYAVYNSIVRKLNHAKMFATFTLPDATAHPIWTRFDKLGGNLHQYTFLFNEFGEGRHAIRFQKLLTVEDGVAKEVDDVTVPISMSAQLDDLLPRDPHELVALYFQDYGAEQHLAGEFGGAKIQYRRDQLNHLHARRGARDVYLNLSVRVQSQSEARGERRPPYAAVFRLVGDNHRAFVHFDKLSDYLAEHPDDGKLGSEGLLSGLRVMSVDLGLRTSASISVFRVARKDELKPNSEGRVPFCFPIEGNENLVAVHERSQLLKLPGETESKDLRAIREERQRTLRQLRTQLAYLRLLVRCGSEDVGRRERSWAKLIEQPMDANQMTPDWREAFEDELQKLKSLYGICGDREWTEAVYESVRRVWRHMGKQVRDWRKDVRSGERPKIRGYQKDVVGGNSIEQIEYLERQYKFLKSWSFFGKVSGQVIRAEKGSRFAITLREHIDHAKEDRLKKLADRIIMEALGYVYALDDERGKGKWVAKYPPCQLILLEELSEYQFNNDRPPSENNQLMQWSHRGVFQELLNQAQVHDLLVGTMYAAFSSRFDARTGAPGIRCRRVPARCARCRKKQKDNKQWEKNKKRGLFKCEGCPLRADDLIPTGEGEFFVSPFSAEEGDFHQIHADLNAAQNLQRRLWSDFDISQIRLRCDWGEVDGEPVLIPRTTGKRTADSYGNKVFYTKTGVTYYERERGKKRRKVFAQEELSEEEAELLVEADEAREKSVVLMRDPSGIINRGDWTRQKEFWSMVNQRIEGYLVKQIRSRVRLQESACENTGDI

SEQ ID NO: 6 - protein, 35 aa, synthetic construct
CFNCGKEGHTARNCRAPRKKGCWKCGKEGHNMKDC

SEQ ID NO: 7 - protein, 1138 aa, synthetic construct
MAVKSMKVKLRLDNMPEIRAGLWKLHTEVNAGVRYYTEWLSLLRQENLYRRSPNGDGEQECYKTAEECKAELLERLRARQVENGHCGPAGSDDELLQLARQLYELLVPQAIGAKGDAQQIARKFLSPLADKDAVGGLGIAKAGNKPRWVRMREAGEPGWEEEKAKAEARKSTDRTADVLRALADFGLKPLMRVYTDSDMSSVQWKPLRKGQAVRTWDRDMFQQAIERMMSWESWNQRVGEAYAKLVEQKSRFEQKNFVGQEHLVQLVNQLQQDMKEASHGLESKEQTAHYLTGRALRGSDKVFEKWEKLDPDAPFDLYDTEIKNVQRRNTRRFGSHDLFAKLAEPKYQALWREDASFLTRYAVYNSIVRKLNHAKMFATFTLPDATAHPIWTRFDKLGGNLHQYTFLFNEFGEGRHAIRFQKLLTVEDGVAKEVDDVTVPISMSAQLDDLLPRDPHELVALYFQDYGAEQHLAGEFGGAKIQYRRDQLNHLHARRGARDVYLNLSVRVQSQSEARGERRPPYAAVFRLVGDNHRAFVHFDKLSDYLAEHPDDGKLGSEGLLSGLRVMSVDLGLRTSASISVFRVARKDELKPNSEGRVPFCFPIEGNENLVAVHERSQLLKLPGETESKDLRAIREERQRTLRQLRTQLAYLRLLVRCGSEDVGRRERSWAKLIEQPMDANQMTPDWREAFEDELQKLKSLYGICGDREWTEAVYESVRRVWRHMGKQVRDWRKDVRSGERPKIRGYQKDVVGGNSIEQIEYLERQYKFLKSWSFFGKVSGQVIRAEKGSRFAITLREHIDHAKEDRLKKLADRIIMEALGYVYALDDERGKGKWVAKYPPCQLILLEELSEYQFNNDRPPSENNQLMQWSHRGVFQELLNQAQVHDLLVGTMYAAFSSRFDARTGAPGIRCRRVPARCFNCGKEGHTARNCRAPRKKGCWKCGKEGHNMKDCPLRADDLIPTGEGEFFVSPFSAEEGDFHQIHADLNAAQNLQRRLWSDFDISQIRLRCDWGEVDGEPVLIPRTTGKRTADSYGNKVFYTKTGVTYYERERGKKRRKVFAQEELSEEEAELLVEADEAREKSVVLMRDPSGIINRGDWTRQKEFWSMVNQRIEGYLVKQIRSRVRLQESACENTGDI

SEQ ID NO: 8 - protein, 102 aa, synthetic construct
SQRPGAHLTVKKIFVGGIKEDTEEHHLRDYFEQYGKIEVIEIMTDRGSGKKRGFAFVTFDDHDSVDKIVIQKYHTVNGHNCEVRKALSKQEMASASSSQRGR

SEQ ID NO: 9 - protein, 1205 aa, synthetic construct
MAVKSMKVKLRLDNMPEIRAGLWKLHTEVNAGVRYYTEWLSLLRQENLYRRSPNGDGEQECYKTAEECKAELLERLRARQVENGHCGPAGSDDELLQLARQLYELLVPQAIGAKGDAQQIARKFLSPLADKDAVGGLGIAKAGNKPRWVRMREAGEPGWEEEKAKAEARKSTDRTADVLRALADFGLKPLMRVYTDSDMSSVQWKPLRKGQAVRTWDRDMFQQAIERMMSWESWNQRVGEAYAKLVEQKSRFEQKNFVGQEHLVQLVNQLQQDMKEASHGLESKEQTAHYLTGRALRGSDKVFEKWEKLDPDAPFDLYDTEIKNVQRRNTRRFGSHDLFAKLAEPKYQALWREDASFLTRYAVYNSIVRKLNHAKMFATFTLPDATAHPIWTRFDKLGGNLHQYTFLFNEFGEGRHAIRFQKLLTVEDGVAKEVDDVTVPISMSAQLDDLLPRDPHELVALYFQDYGAEQHLAGEFGGAKIQYRRDQLNHLHARRGARDVYLNLSVRVQSQSEARGERRPPYAAVFRLVGDNHRAFVHFDKLSDYLAEHPDDGKLGSEGLLSGLRVMSVDLGLRTSASISVFRVARKDELKPNSEGRVPFCFPIEGNENLVAVHERSQLLKLPGETESKDLRAIREERQRTLRQLRTQLAYLRLLVRCGSEDVGRRERSWAKLIEQPMDANQMTPDWREAFEDELQKLKSLYGICGDREWTEAVYESVRRVWRHMGKQVRDWRKDVRSGERPKIRGYQKDVVGGNSIEQIEYLERQYKFLKSWSFFGKVSGQVIRAEKGSRFAITLREHIDHAKEDRLKKLADRIIMEALGYVYALDDERGKGKWVAKYPPCQLILLEELSEYQFNNDRPPSENNQLMQWSHRGVFQELLNQAQVHDLLVGTMYAAFSSRFDARTGAPGIRCRRVPARSQRPGAHLTVKKIFVGGIKEDTEEHHLRDYFEQYGKIEVIEIMTDRGSGKKRGFAFVTFDDHDSVDKIVIQKYHTVNGHNCEVRKALSKQEMASASSSQRGRPLRADDLIPTGEGEFFVSPFSAEEGDFHQIHADLNAAQNLQRRLWSDFDISQIRLRCDWGEVDGEPVLIPRTTGKRTADSYGNKVFYTKTGVTYYERERGKKRRKVFAQEELSEEEAELLVEADEAREKSVVLMRDPSGIINRGDWTRQKEFWSMVNQRIEGYLVKQIRSRVRLQESACENTGDI

SEQ ID NO: 10 - protein, 29 aa, synthetic construct
CAREQNPEPFPWWLNKFVAEHKLDGCPLR

SEQ ID NO: 11 - protein, 6 aa, synthetic construct
GGGGGG

SEQ ID NO: 12 - protein, 1109 aa, synthetic construct
MAVKSMKVKLRLDNMPEIRAGLWKLHTEVNAGVRYYTEWLSLLRQENLYRRSPNGDGEQECYKTAEECKAELLERLRARQVENGHCGPAGSDDELLQLARQLYELLVPQAIGAKGDAQQIARKFLSPLADKDAVGGLGIAKAGNKPRWVRMREAGEPGWEEEKAKAEARKSTDRTADVLRALADFGLKPLMRVYTDSDMSSVQWKPLRKGQAVRTWDRDMFQQAIERMMSWESWNQRVGEAYAKLVEQKSRFEQKNFVGQEHLVQLVNQLQQDMKEASHGLESKEQTAHYLTGRALRGSDKVFEKWEKLDPDAPFDLYDTEIKNVQRRNTRRFGSHDLFAKLAEPKYQALWREDASFLTRYAVYNSIVRKLNHAKMFATFTLPDATAHPIWTRFDKLGGNLHQYTFLFNEFGEGRHAIRFQKLLTVEDGVAKEVDDVTVPISMSAQLDDLLPRDPHELVALYFQDYGAEQHLAGEFGGAKIQYRRDQLNHLHARRGARDVYLNLSVRVQSQSEARGERRPPYAAVFRLVGDNHRAFVHFDKLSDYLAEHPDDGKLGSEGLLSGLRVMSVDLGLRTSASISVFRVARKDELKPNSEGRVPFCFPIEGNENLVAVHERSQLLKLPGETESKDLRAIREERQRTLRQLRTQLAYLRLLVRCGSEDVGRRERSWAKLIEQPMDANQMTPDWREAFEDELQKLKSLYGICGDREWTEAVYESVRRVWRHMGKQVRDWRKDVRSGERPKIRGYQKDVVGGNSIEQIEYLERQYKFLKSWSFFGKVSGQVIRAEKGSRFAITLREHIDHAKEDRLKKLADRIIMEALGYVYALDDERGKGKWVAKYPPCQLILLEELSEYQFNNDRPPSENNQLMQWSHRGVFQELLNQAQVHDLLVGTMYAAFSSRFDARTGAPGIRCRRVPARGGGGGGPLRADDLIPTGEGEFFVSPFSAEEGDFHQIHADLNAAQNLQRRLWSDFDISQIRLRCDWGEVDGEPVLIPRTTGKRTADSYGNKVFYTKTGVTYYERERGKKRRKVFAQEELSEEEAELLVEADEAREKSVVLMRDPSGIINRGDWTRQKEFWSMVNQRIEGYLVKQIRSRVRLQESACENTGDI

SEQ ID NO: 13 - protein, 60 aa, synthetic construct
RFDARTGAPGIRCRRVPARCAREQNPEPFPWWLNKFVAEHKLDGCPLRADDLIPTGEGEF

SEQ ID NO: 14 - protein, 46 aa, synthetic construct
RGMRVVTVPYLASSKVCAECRKKQKDNKQWEKNKKRGLFKCEGCGS

SEQ ID NO: 15 - RNA, 103 nt, synthetic construct
  source 1..103: mol_type = other RNA
gtctaaaggacagattttcaacgggtgtgccaatggccactttccaggtggcaaagcccgttgaacttcaagcgaagtggcacactcaatacttgagcacact

SEQ ID NO: 16 - DNA, 946 bp, synthetic construct
  source 1..946: mol_type = other DNA
taatacgactcactatagggcttcacctgatgctgttacagcgtataatggttatcttacttcttcttctaaaacacctgaagaacattttattgaaaccatctcacttgctggttcctataaagattggtcctattctggacaatctacacaactaggtatagaatttcttaagagaggtgataaaagtgtatattacactagtaatcctaccacattccacctagatggtgaagttatcacctttgacaatcttaagacacttctttctttgagagaagtgaggactattaaggtgtttacaacagtagacaacattaacctccacacgcaagttgtggacatgtcaatgacatatgggtgttgctatgcctaatctttacaaaatgcaaagaatgctattagaaaagtgtgaccttcaaaattatggtgatagtgcaacattacctaaaggcataatgatgaatgtcgcaaaatatactcaactgtgtcaatatttaaacacattaacattagctgtaccctataatatgagagttatacattttacacttaacggtctttggcttgatgacgtagtttactgtccaagacatgtgatctgcacctctgaagacatgcttaaccctaattatgaagaaaggttgatacagccaatcctaagacacctaagtataagtttgttcgcattcaaccaggacagactttttcagtgttagcttgttacaatggttcaccatctggtgtttaccaatgtgctatgaggcccaatttcactattaagggttcattccttgtttctatagattagctaatgagtgtgctcaagtattgagtgaaatggtcatgtgtggcggttcactatatgttaaaccaggtggaacctcatcaggagatgccacaactgcttatgctaatagtgtttttaacatttgtcaagctgtca

SEQ ID NO: 17 - RNA, 19 nt, synthetic construct
  source 1..19: mol_type = other RNA
tttagcaggattcaggttt

SEQ ID NO: 18 - RNA, 39 nt, synthetic construct
  source 1..39: mol_type = other RNA
catattgacgcatacaaaacattcccaccaacagagcct

SEQ ID NO: 19 - RNA, 10 nt, synthetic construct
  source 1..10: mol_type = other RNA
cccccccccc

SEQ ID NO: 20 - DNA, 33 bp, synthetic construct
  source 1..33: mol_type = other DNA
ttacttcttcttctaaaacacctgaagaacatt

SEQ ID NO: 21 - DNA, 33 bp, synthetic construct
  source 1..33: mol_type = other DNA
gtgtagattgtccagaataggaccaatctttat